European Patent Specification EP 3 824 081 B1, published July 26, 2023. Title: Linalool Synthases. Applicant: C3 Bio-Technologies Limited. The sequence listing filed with the application follows.

SEQUENCE LISTING (39 sequences)

SEQ ID NO: 1 - protein, 329 aa, Artificial Sequence
  Linalool synthase from Streptomyces clavuligerus (L72 and V214 shaded)
MQEFEFAVPAPSRVSPDLARARARHLDWVHAMDLVRGEEARRRYEFSCVADIGAYGYPHATGADLDLCVDVLGWTFLFDDQFDAGDGRERDALAVCAELTDLLWKGTAATAASPPIVVAFSDCWERMRAGMSDAWRRRTVHEWVDYLAGWPTKLADRAHGAVLDPAAHLRARHRTICCRPLFALAERVGGYEVPRRAWHSSRLDGMRFTTSDAVIGMNELHSFEKDRAQGHANLVLSLVHHGGLTGPEAVTRVCDLVQGSIESFLRLRSGLPELGRALGVEGAVLDRYADALSAFCRGYHDWGRGASRYTTRDHPGDLGLENLVARSSG

SEQ ID NO: 2 - protein, 329 aa, Artificial Sequence
  Linalool synthase variant bLinS-L72M
MQEFEFAVPAPSRVSPDLARARARHLDWVHAMDLVRGEEARRRYEFSCVADIGAYGYPHATGADLDLCVDVMGWTFLFDDQFDAGDGRERDALAVCAELTDLLWKGTAATAASPPIVVAFSDCWERMRAGMSDAWRRRTVHEWVDYLAGWPTKLADRAHGAVLDPAAHLRARHRTICCRPLFALAERVGGYEVPRRAWHSSRLDGMRFTTSDAVIGMNELHSFEKDRAQGHANLVLSLVHHGGLTGPEAVTRVCDLVQGSIESFLRLRSGLPELGRALGVEGAVLDRYADALSAFCRGYHDWGRGASRYTTRDHPGDLGLENLVARSSG

SEQ ID NO: 3 - protein, 329 aa, Artificial Sequence
  Linalool synthase variant bLinS-V214L
MQEFEFAVPAPSRVSPDLARARARHLDWVHAMDLVRGEEARRRYEFSCVADIGAYGYPHATGADLDLCVDVLGWTFLFDDQFDAGDGRERDALAVCAELTDLLWKGTAATAASPPIVVAFSDCWERMRAGMSDAWRRRTVHEWVDYLAGWPTKLADRAHGAVLDPAAHLRARHRTICCRPLFALAERVGGYEVPRRAWHSSRLDGMRFTTSDALIGMNELHSFEKDRAQGHANLVLSLVHHGGLTGPEAVTRVCDLVQGSIESFLRLRSGLPELGRALGVEGAVLDRYADALSAFCRGYHDWGRGASRYTTRDHPGDLGLENLVARSSG

SEQ ID NO: 4 - protein, 329 aa, Artificial Sequence
  Linalool synthase variant bLinS-V214I
MQEFEFAVPAPSRVSPDLARARARHLDWVHAMDLVRGEEARRRYEFSCVADIGAYGYPHATGADLDLCVDVLGWTFLFDDQFDAGDGRERDALAVCAELTDLLWKGTAATAASPPIVVAFSDCWERMRAGMSDAWRRRTVHEWVDYLAGWPTKLADRAHGAVLDPAAHLRARHRTICCRPLFALAERVGGYEVPRRAWHSSRLDGMRFTTSDAIIGMNELHSFEKDRAQGHANLVLSLVHHGGLTGPEAVTRVCDLVQGSIESFLRLRSGLPELGRALGVEGAVLDRYADALSAFCRGYHDWGRGASRYTTRDHPGDLGLENLVARSSG

SEQ ID NO: 5 - protein, 329 aa, Artificial Sequence
  Linalool synthase variant bLinS-L72M-V214I
MQEFEFAVPAPSRVSPDLARARARHLDWVHAMDLVRGEEARRRYEFSCVADIGAYGYPHATGADLDLCVDVMGWTFLFDDQFDAGDGRERDALAVCAELTDLLWKGTAATAASPPIVVAFSDCWERMRAGMSDAWRRRTVHEWVDYLAGWPTKLADRAHGAVLDPAAHLRARHRTICCRPLFALAERVGGYEVPRRAWHSSRLDGMRFTTSDAIIGMNELHSFEKDRAQGHANLVLSLVHHGGLTGPEAVTRVCDLVQGSIESFLRLRSGLPELGRALGVEGAVLDRYADALSAFCRGYHDWGRGASRYTTRDHPGDLGLENLVARSSG

SEQ ID NO: 6 - protein, 329 aa, Artificial Sequence
  Linalool synthase variant bLinS-L72M-V214L
MQEFEFAVPAPSRVSPDLARARARHLDWVHAMDLVRGEEARRRYEFSCVADIGAYGYPHATGADLDLCVDVMGWTFLFDDQFDAGDGRERDALAVCAELTDLLWKGTAATAASPPIVVAFSDCWERMRAGMSDAWRRRTVHEWVDYLAGWPTKLADRAHGAVLDPAAHLRARHRTICCRPLFALAERVGGYEVPRRAWHSSRLDGMRFTTSDALIGMNELHSFEKDRAQGHANLVLSLVHHGGLTGPEAVTRVCDLVQGSIESFLRLRSGLPELGRALGVEGAVLDRYADALSAFCRGYHDWGRGASRYTTRDHPGDLGLENLVARSSG

SEQ ID NO: 7 - protein, 355 aa, Artificial Sequence
  Linalool synthase from Streptomyces clavuligerus with leader sequence
MKHHHHHHPMSDYDIPTTENLYFQGAMQEFEFAVPAPSRVSPDLARARARHLDWVHAMDLVRGEEARRRYEFSCVADIGAYGYPHATGADLDLCVDVLGWTFLFDDQFDAGDGRERDALAVCAELTDLLWKGTAATAASPPIVVAFSDCWERMRAGMSDAWRRRTVHEWVDYLAGWPTKLADRAHGAVLDPAAHLRARHRTICCRPLFALAERVGGYEVPRRAWHSSRLDGMRFTTSDAVIGMNELHSFEKDRAQGHANLVLSLVHHGGLTGPEAVTRVCDLVQGSIESFLRLRSGLPELGRALGVEGAVLDRYADALSAFCRGYHDWGRGASRYTTRDHPGDLGLENLVARSSG

SEQ ID NO: 8 - protein, 355 aa, Artificial Sequence
  Linalool synthase variant bLinS-L72M with leader sequence
MKHHHHHHPMSDYDIPTTENLYFQGAMQEFEFAVPAPSRVSPDLARARARHLDWVHAMDLVRGEEARRRYEFSCVADIGAYGYPHATGADLDLCVDVMGWTFLFDDQFDAGDGRERDALAVCAELTDLLWKGTAATAASPPIVVAFSDCWERMRAGMSDAWRRRTVHEWVDYLAGWPTKLADRAHGAVLDPAAHLRARHRTICCRPLFALAERVGGYEVPRRAWHSSRLDGMRFTTSDAVIGMNELHSFEKDRAQGHANLVLSLVHHGGLTGPEAVTRVCDLVQGSIESFLRLRSGLPELGRALGVEGAVLDRYADALSAFCRGYHDWGRGASRYTTRDHPGDLGLENLVARSSG

SEQ ID NO: 9 - protein, 355 aa, Artificial Sequence
  Linalool synthase variant bLinS-V214L with leader sequence
MKHHHHHHPMSDYDIPTTENLYFQGAMQEFEFAVPAPSRVSPDLARARARHLDWVHAMDLVRGEEARRRYEFSCVADIGAYGYPHATGADLDLCVDVLGWTFLFDDQFDAGDGRERDALAVCAELTDLLWKGTAATAASPPIVVAFSDCWERMRAGMSDAWRRRTVHEWVDYLAGWPTKLADRAHGAVLDPAAHLRARHRTICCRPLFALAERVGGYEVPRRAWHSSRLDGMRFTTSDALIGMNELHSFEKDRAQGHANLVLSLVHHGGLTGPEAVTRVCDLVQGSIESFLRLRSGLPELGRALGVEGAVLDRYADALSAFCRGYHDWGRGASRYTTRDHPGDLGLENLVARSSG

SEQ ID NO: 10 - protein, 355 aa, Artificial Sequence
  Linalool synthase variant bLinS-V214I with leader sequence
MKHHHHHHPMSDYDIPTTENLYFQGAMQEFEFAVPAPSRVSPDLARARARHLDWVHAMDLVRGEEARRRYEFSCVADIGAYGYPHATGADLDLCVDVLGWTFLFDDQFDAGDGRERDALAVCAELTDLLWKGTAATAASPPIVVAFSDCWERMRAGMSDAWRRRTVHEWVDYLAGWPTKLADRAHGAVLDPAAHLRARHRTICCRPLFALAERVGGYEVPRRAWHSSRLDGMRFTTSDAIIGMNELHSFEKDRAQGHANLVLSLVHHGGLTGPEAVTRVCDLVQGSIESFLRLRSGLPELGRALGVEGAVLDRYADALSAFCRGYHDWGRGASRYTTRDHPGDLGLENLVARSSG

SEQ ID NO: 11 - protein, 355 aa, Artificial Sequence
  Linalool synthase variant bLinS-L72M-V214I with leader sequence
MKHHHHHHPMSDYDIPTTENLYFQGAMQEFEFAVPAPSRVSPDLARARARHLDWVHAMDLVRGEEARRRYEFSCVADIGAYGYPHATGADLDLCVDVMGWTFLFDDQFDAGDGRERDALAVCAELTDLLWKGTAATAASPPIVVAFSDCWERMRAGMSDAWRRRTVHEWVDYLAGWPTKLADRAHGAVLDPAAHLRARHRTICCRPLFALAERVGGYEVPRRAWHSSRLDGMRFTTSDAIIGMNELHSFEKDRAQGHANLVLSLVHHGGLTGPEAVTRVCDLVQGSIESFLRLRSGLPELGRALGVEGAVLDRYADALSAFCRGYHDWGRGASRYTTRDHPGDLGLENLVARSSG

SEQ ID NO: 12 - protein, 355 aa, Artificial Sequence
  Linalool synthase variant bLinS-L72M-V214L with leader sequence
MKHHHHHHPMSDYDIPTTENLYFQGAMQEFEFAVPAPSRVSPDLARARARHLDWVHAMDLVRGEEARRRYEFSCVADIGAYGYPHATGADLDLCVDVMGWTFLFDDQFDAGDGRERDALAVCAELTDLLWKGTAATAASPPIVVAFSDCWERMRAGMSDAWRRRTVHEWVDYLAGWPTKLADRAHGAVLDPAAHLRARHRTICCRPLFALAERVGGYEVPRRAWHSSRLDGMRFTTSDALIGMNELHSFEKDRAQGHANLVLSLVHHGGLTGPEAVTRVCDLVQGSIESFLRLRSGLPELGRALGVEGAVLDRYADALSAFCRGYHDWGRGASRYTTRDHPGDLGLENLVARSSG

SEQ ID NO: 13 - protein, 26 aa, Artificial Sequence
  Linalool synthase leader sequence
MKHHHHHHPMSDYDIPTTENLYFQGA

SEQ ID NO: 14 - DNA, 33 bp, Artificial Sequence
  Primer bLinS-L72F_fw
ctgtgtgttgatgttttcggttggacctttctg

SEQ ID NO: 15 - DNA, 33 bp, Artificial Sequence
  Primer bLinS-L72M_fw
ctgtgtgttgatgttatgggttggacctttctg

SEQ ID NO: 16 - DNA, 33 bp, Artificial Sequence
  Primer bLinS-L72I_fw
ctgtgtgttgatgttattggttggacctttctg

SEQ ID NO: 17 - DNA, 33 bp, Artificial Sequence
  Primer bLinS-L72N_fw
ctgtgtgttgatgttaccggttggacctttctg

SEQ ID NO: 18 - DNA, 33 bp, Artificial Sequence
  Primer bLinS-L72Q_fw
ctgtgtgttgatgttcagggttggacctttctg

SEQ ID NO: 19 - DNA, 34 bp, Artificial Sequence
  Primer bLinS-T75F_fw
gatgttctgggttggttctttctgtttgatgatc

SEQ ID NO: 20 - DNA, 34 bp, Artificial Sequence
  Primer bLinS-T75M_fw
gatgttctgggttggatgtttctgtttgatgatc

SEQ ID NO: 21 - DNA, 31 bp, Artificial Sequence
  Primer bLinS-I176F_fw
gctcgccatcgtaccttttgttgtcgtccgc

SEQ ID NO: 22 - DNA, 31 bp, Artificial Sequence
  Primer bLinS-C177F_fw
catcgtaccatttgttttcgtccgctgtttg

SEQ ID NO: 23 - DNA, 31 bp, Artificial Sequence; identical to SEQ ID NO: 22
  Primer bLinS-C178F_fw

SEQ ID NO: 24 - DNA, 31 bp, Artificial Sequence
  Primer bLinS-C178M_fw
catcgtaccatttgtatgcgtccgctgtttg

SEQ ID NO: 25 - DNA, 30 bp, Artificial Sequence
  Primer bLinS-V214F_fw
ccaccagtgatgcatttattggtatgaatg

SEQ ID NO: 26 - DNA, 30 bp, Artificial Sequence
  Primer bLinS-V214L_fw
ccaccagtgatgcactgattggtatgaatg

SEQ ID NO: 27 - DNA, 30 bp, Artificial Sequence
  Primer bLinS-V214I_fw
ccaccagtgatgcaattattggtatgaatg

SEQ ID NO: 28 - DNA, 30 bp, Artificial Sequence
  Primer bLinS-V214M_fw
ccaccagtgatgcaatgattggtatgaatg

SEQ ID NO: 29 - DNA, 30 bp, Artificial Sequence
  Primer bLinS-V214S_fw
ccaccagtgatgcaagtattggtatgaatg

SEQ ID NO: 30 - DNA, 28 bp, Artificial Sequence
  Primer bLinS-F295W_fw
gcactgagcgcatggtgtcgtggttatc

SEQ ID NO: 31 - DNA, 28 bp, Artificial Sequence
  Primer bLinS-F295Y_fw
gcactgagcgcatattgtcgtggttatc

SEQ ID NO: 32 - protein, 5 aa, Artificial Sequence
  aspartate-rich motif
  misc_feature (3)..(4): Xaa can be any naturally occurring amino acid
DDXXD

SEQ ID NO: 33 - protein, 5 aa, Artificial Sequence
  aspartate-rich motif
  misc_feature (3)..(4): Xaa can be any naturally occurring amino acid
DDXXE

SEQ ID NO: 34 - protein, 6 aa, Artificial Sequence
  aspartate-rich motif
  misc_feature (3)..(5): Xaa can be any naturally occurring amino acid
DDXXXD

SEQ ID NO: 35 - protein, 6 aa, Artificial Sequence
  aspartate-rich motif
  misc_feature (3)..(5): Xaa can be any naturally occurring amino acid
DDXXXE

SEQ ID NO: 36 - protein, 9 aa, Artificial Sequence
  NSE triad
  misc_feature (3)..(4): Xaa can be any naturally occurring amino acid
  misc_feature (6)..(7): Xaa can be any naturally occurring amino acid
NDXXSXXRE

SEQ ID NO: 37 - protein, 9 aa, Artificial Sequence
  NSE triad
  misc_feature (3)..(4): Xaa can be any naturally occurring amino acid
  misc_feature (6)..(7): Xaa can be any naturally occurring amino acid
NDXXSXXRD

SEQ ID NO: 38 - protein, 9 aa, Artificial Sequence
  NSE triad
  misc_feature (3)..(4): Xaa can be any naturally occurring amino acid
  misc_feature (6)..(7): Xaa can be any naturally occurring amino acid
NDXXSXXKE

SEQ ID NO: 39 - protein, 9 aa, Artificial Sequence
  NSE triad
  misc_feature (3)..(4): Xaa can be any naturally occurring amino acid
  misc_feature (6)..(7): Xaa can be any naturally occurring amino acid
NDXXSXXKD